European Patent Application EP 4 385 997 A1, published June 19, 2024. Title: CHITINOPEPTINS, THEIR USE AND RECOMBINANT SYNTHESIS IN ORGANISMS FOR PLANT PROTECTION. Applicant: Fraunhofer-Gesellschaft zur Förderung der angewandten Forschung e.V. Application EP. The sequence listing filed with the application follows.

SEQUENCE LISTING (12 sequences)

SEQ ID NO: 1 - protein, 15 aa, synthetic construct
  SITE 1: note = absent or L-2,3-Diaminopropionic acid
  MOD_RES 2: note = N-Methyl-L-valine
  SITE 3: note = D-Allo-threonine
  SITE 4: note = D-Alanine
  MOD_RES 5: note = (2S,3S)-3-hydroxyaspartic acid
  MOD_RES 6: note = (2S,3R)-3-hydroxyphenylalanine
  SITE 7: note = D-allo-isoleucine
  SITE 9: note = D-Lysine
  SITE 10: note = L-2,3-Diaminopropionic acid
  SITE 11: note = D-Valine, D-allo-isoleucine, or D-Leucine
  MOD_RES 12: note = (2S,3S)-3-hydroxyaspartic acid
  MOD_RES 14: note = (2S,3S)-3-hydroxyaspartic acid
  MOD_RES 15: note = (2S,3R)-3-hydroxyisoleucine
  CROSSLNK 3..15: note = Side chain of D-Allo-threonine linked to C-terminal carboxyl group of (2S,3R)-3-hydroxyisoleucine via a ester bond (D-Allo-threonine-(2S,3R)-3-hydroxyisoleucine)
  VARIANT 5: note = In a variant, (2S,3S)-3-hydroxyaspartic acid is connected via its side chain carboxyl group to the amino group of the (2S,3R)-3-hydroxyphenylalanine
  VARIANT 9: note = In a variant, D-Lysine is connected via its side chain amino group to the carboxyl group of the preceding L-Serine
  VARIANT 10: note = In a variant, L-2,3-Diaminopropionic acid is connected via its side chain amino group to the carboxyl group of the preceding D-Lysine
  VARIANT 12: note = In a variant, (2S,3S)-3-hydroxyaspartic acid is connected via its side chain carboxyl group to the amino group of the L-Leucine
  VARIANT 14: note = In a variant, (2S,3S)-3-hydroxyaspartic acid is connected via its side chain carboxyl group to the amino group of the (2S,3R)-3-hydroxyisoleucine
XVTADFISKXXDLDI

SEQ ID NO: 2 - protein, 13 aa, synthetic construct
  SITE 1: note = D-Allo-threonine
  SITE 2: note = D-Alanine
  MOD_RES 3: note = (2S,3S)-3-hydroxyaspartic acid
  MOD_RES 4: note = (2S,3R)-3-hydroxyphenylalanine
  SITE 5: note = D-allo-isoleucine
  SITE 7: note = D-Lysine
  SITE 8: note = L-2,3-Diaminopropionic acid
  SITE 9: note = D-Valine, D-allo-isoleucine, or D-Leucine
  MOD_RES 10: note = (2S,3S)-3-hydroxyaspartic acid
  MOD_RES 12: note = (2S,3S)-3-hydroxyaspartic acid
  MOD_RES 13: note = (2S,3R)-3-hydroxyisoleucine
  CROSSLNK 1..13: note = Side chain of D-Allo-threonine linked to C-terminal carboxyl group of (2S,3R)-3-hydroxyisoleucine via a ester bond (D-Allo-threonine-(2S,3R)-3-hydroxyisoleucine)
  VARIANT 3: note = In a variant, (2S,3S)-3-hydroxyaspartic acid is connected via its side chain carboxyl group to the amino group of the (2S,3R)-3-hydroxyphenylalanine
  VARIANT 7: note = In a variant, D-Lysine is connected via its side chain amino group to the carboxyl group of the preceding L-Serine
  VARIANT 8: note = In a variant, L-2,3-Diaminopropionic acid is connected via its side chain amino group to the carboxyl group of the preceding D-Lysine
  VARIANT 10: note = In a variant, (2S,3S)-3-hydroxyaspartic acid is connected via its side chain carboxyl group to the amino group of the L-Leucine
  VARIANT 12: note = In a variant, (2S,3S)-3-hydroxyaspartic acid is connected via its side chain carboxyl group to the amino group of the (2S,3R)-3-hydroxyisoleucine
TADFISKXXDLDI

SEQ ID NO: 3 - protein, 9 aa, synthetic construct
  SITE 1: note = absent or L-2,3-Diaminopropionic acid
  MOD_RES 2: note = N-Methyl-L-valine
  SITE 3: note = D-Allo-threonine; note = Side chain of D-Allo-threonine linked to C-terminal carboxylic acid group of (2S,3R)-3-hydroxyisoleucine of another sequence (SEQ ID NO. 4) via a ester bond (D-Allo-threonine-(2S,3R)-3-hydroxyisoleucine)
  SITE 4: note = D-Alanine
  MOD_RES 5: note = (2S,3S)-3-hydroxyaspartic acid
  MOD_RES 6: note = (2S,3R)-3-hydroxyphenylalanine
  SITE 7: note = D-allo-isoleucine
  SITE 9: note = Carboxy-terminus of D-Lysine is linked to the side chain amino group of L-2,3-Diaminopropionic acid of another sequence (SEQ ID NO. 4) via carboxamide bond (D-Lysine-L-2,3-Diaminopropionic acid); note = D-Lysine
XVTADFISK

SEQ ID NO: 4 - protein, 6 aa, synthetic construct
  SITE 1: note = Side chain of L-2,3-Diaminopropionic acid linked to the C-terminal carboxyl group of D-Lysine of another sequence (SEQ ID NO. 3) via carboxamide bond (D-Lysine-L-2,3-Diaminopropionic acid); note = L-2,3-Diaminopropionic acid
  SITE 2: note = D-Valine, D-allo-isoleucine, or D-Leucine
  MOD_RES 3: note = (2S,3S)-3-hydroxyaspartic acid
  MOD_RES 5: note = (2S,3S)-3-hydroxyaspartic acid
  MOD_RES 6: note = (2S,3R)-3-hydroxyisoleucine
  SITE 6: note = C-terminal carboxylic acid group of (2S,3R)-3-hydroxyisoleucine linked to side chain of D-Allo-threonine of another sequence (SEQ ID NO. 3) via a ester bond (D-Allo-threonine-(2S,3R)-3-hydroxyisoleucine)
XXDLDI

SEQ ID NO: 5 - protein, 15 aa, synthetic construct
  SITE 1: note = absent or L-2,3-Diaminopropionic acid
  MOD_RES 2: note = N-Methyl-L-valine
  SITE 3: note = D-Allo-threonine
  SITE 4: note = D-Alanine
  MOD_RES 5: note = (2S,3S)-3-hydroxyaspartic acid
  MOD_RES 6: note = (2S,3R)-3-hydroxyphenylalanine
  SITE 7: note = D-allo-isoleucine
  SITE 9: note = D-Lysine
  SITE 10: note = L-2,3-Diaminopropionic acid
  SITE 11: note = D-Valine, D-allo-isoleucine, or D-Leucine
  MOD_RES 12: note = (2S,3S)-3-hydroxyaspartic acid
  MOD_RES 14: note = (2S,3S)-3-hydroxyaspartic acid
  MOD_RES 15: note = (2S,3R)-3-hydroxyisoleucine
  CROSSLNK 3..15: note = Side chain of D-Allo-threonine linked to C-terminal carboxyl group of (2S,3R)-3-hydroxyisoleucine via a ester bond (D-Allo-threonine-(2S,3R)-3-hydroxyisoleucine)
XVTADFISKXXDLDI

SEQ ID NO: 6 - protein, 14 aa, Chitinophaga eiseniae
  SITE 2: note = D-Allo-threonine
  SITE 3: note = D-Alanine
  MOD_RES 4: note = (2S,3S)-3-hydroxyaspartic acid
  MOD_RES 5: note = (2S,3R)-3-hydroxyphenylalanine
  SITE 6: note = D-allo-isoleucine
  SITE 8: note = D-Lysine
  SITE 9: note = L-2,3-Diaminopropionic acid
  SITE 10: note = D-Leucine
  MOD_RES 11: note = (2S,3S)-3-hydroxyaspartic acid
  MOD_RES 13: note = (2S,3S)-3-hydroxyaspartic acid
  MOD_RES 14: note = (2S,3R)-3-hydroxyisoleucine
  MOD_RES 1: note = N-Methyl-L-valine
  CROSSLNK 2..14: note = Side chain of D-Allo-threonine linked to C-terminal carboxylic acid group of (2S,3R)-3-hydroxyisoleucine via a ester bond (D-Allo-threonine-(2S,3R)-3-hydroxyisoleucine)
VTADFISKXLDLDI

SEQ ID NO: 7 - protein, 15 aa, Chitinophaga flava
  SITE 1: note = L-2,3-Diaminopropionic acid
  MOD_RES 2: note = N-Methyl-L-valine
  SITE 3: note = D-Allo-threonine
  SITE 4: note = D-Alanine
  MOD_RES 5: note = (2S,3S)-3-hydroxyaspartic acid
  MOD_RES 6: note = (2S,3R)-3-hydroxyphenylalanine
  SITE 7: note = D-allo-isoleucine
  SITE 9: note = D-Lysine
  SITE 10: note = L-2,3-Diaminopropionic acid
  SITE 11: note = D-allo-isoleucine
  MOD_RES 12: note = (2S,3S)-3-hydroxyaspartic acid
  MOD_RES 14: note = (2S,3S)-3-hydroxyaspartic acid
  MOD_RES 15: note = (2S,3R)-3-hydroxyisoleucine
  CROSSLNK 3..15: note = Side chain of D-Allo-threonine linked to C-terminal carboxyl group of (2S,3R)-3-hydroxyisoleucine via a ester bond (D-Allo-threonine-(2S,3R)-3-hydroxyisoleucine)
XVTADFISKXIDLDI

SEQ ID NO: 8 - protein, 15 aa, Chitinophaga flava
  CROSSLNK 3..15: note = Side chain of D-Allo-threonine linked to C-terminal carboxyl group of (2S,3R)-3-hydroxyisoleucine via a ester bond (D-Allo-threonine-(2S,3R)-3-hydroxyisoleucine)
  SITE 1: note = L-2,3-Diaminopropionic acid
  MOD_RES 2: note = N-Methyl-L-valine
  SITE 3: note = D-Allo-threonine
  SITE 4: note = D-Alanine
  MOD_RES 5: note = (2S,3S)-3-hydroxyaspartic acid
  MOD_RES 6: note = (2S,3R)-3-hydroxyphenylalanine
  SITE 7: note = D-allo-isoleucine
  SITE 9: note = D-Lysine
  SITE 10: note = L-2,3-Diaminopropionic acid
  SITE 11: note = D-Valine
  MOD_RES 12: note = (2S,3S)-3-hydroxyaspartic acid
  MOD_RES 14: note = (2S,3S)-3-hydroxyaspartic acid
  MOD_RES 15: note = (2S,3R)-3-hydroxyisoleucine
XVTADFISKXVDLDI

SEQ ID NO: 9 - protein, 9 aa, Chitinophaga flava
  SITE 1: note = L-2,3-Diaminopropionic acid
  MOD_RES 2: note = N-Methyl-L-valine
  SITE 3: note = Side chain of D-Allo-threonine linked to C-terminal carboxyl group of (2S,3R)-3-hydroxyisoleucine of Chitinopeptine C1 second sequence (SEQ ID NO. 10) via a ester bond (D-Allo-threonine-(2S,3R)-3-hydroxyisoleucine); note = D-Allo-threonine
  SITE 4: note = D-Alanine
  MOD_RES 5: note = (2S,3S)-3-hydroxyaspartic acid
  MOD_RES 6: note = (2S,3R)-3-hydroxyphenylalanine
  SITE 7: note = D-allo-isoleucine
  SITE 9: note = D-Lysine; note = Carboxy-terminus of D-Lysine is linked to the side chain amino group of the N-terminal L-2,3-Diaminopropionic acid of Chitinopeptin C1 second sequence (SEQ ID NO. 10) via carboxamide bond (D-Lysine-L-2,3-Diaminopropinic acid)
XVTADFISK

SEQ ID NO: 10 - protein, 6 aa, Chitinophaga flava
  SITE 1: note = L-2,3-Diaminopropionic acid; note = Side chain of L-2,3-Diaminopropionic acid linked to C-terminal amino acid of Chitinopeptin C1 first sequence (SEQ ID NO. 9) via carboxamide bond (D-Lysine-L-2,3-Diaminopropionic acid)
  SITE 2: note = D-allo-isoleucine
  MOD_RES 3: note = (2S,3S)-3-hydroxyaspartic acid
  MOD_RES 5: note = (2S,3S)-3-hydroxyaspartic acid
  MOD_RES 6: note = (2S,3R)-3-hydroxyisoleucine
  SITE 6: note = C-terminal carboxyl group of (2S,3R)-3-hydroxyisoleucine linked to side chain of D-Allo-threonine of Chitinopeptin C1 first sequence (SEQ ID NO. 9) via a ester bond (D-Allo-threonine-(2S,3R)-3-hydroxyisoleucine)
XIDLDI

SEQ ID NO: 11 - protein, 9 aa, Chitinophaga flava
  SITE 1: note = L-2,3-Diaminopropionic acid
  MOD_RES 2: note = N-Methyl-L-valine
  SITE 3: note = D-Allo-threonine; note = Side chain of D-Allo-threonine linked to C-terminal carboxyl group of (2S,3R)-3-hydroxyisoleucine of Chitinopeptine D1 second sequence (SEQ ID NO. 12) via a ester bond (D-Allo-threonine-(2S,3R)-3-hydroxyisoleucine)
  SITE 4: note = D-Alanine
  MOD_RES 5: note = (2S,3S)-3-hydroxyaspartic acid
  MOD_RES 6: note = (2S,3R)-3-hydroxyphenylalanine
  SITE 7: note = D-allo-isoleucine
  SITE 9: note = Carboxy-terminus of D-Lysine is linked to the side chain amino group of the N-terminal L-2,3-Diaminopropionic acid of Chitinopeptin D1 second sequence (SEQ ID NO. 12) via carboxamide bond (D-Lysine-L-2,3-Diaminopropinic acid); note = D-Lysine
XVTADFISK

SEQ ID NO: 12 - protein, 6 aa, Chitinophaga flava
  SITE 1: note = Side chain of L-2,3-Diaminopropionic acid linked to C-terminal amino acid of Chitinopeptin D1 first sequence (SEQ ID NO. 11) via carboxamide bond (D-Lysine-L-2,3-Diaminopropionic acid); note = L-2,3-Diaminopropionic acid
  SITE 2: note = D-Valine
  MOD_RES 3: note = (2S,3S)-3-hydroxyaspartic acid
  MOD_RES 5: note = (2S,3S)-3-hydroxyaspartic acid
  MOD_RES 6: note = (2S,3R)-3-hydroxyisoleucine
  SITE 6: note = C-terminal carboxyl group of (2S,3R)-3-hydroxyisoleucine linked to side chain of D-Allo-threonine of Chitinopeptin D1 first sequence (SEQ ID NO. 11) via a ester bond (D-Allo-threonine-(2S,3R)-3-hydroxyisoleucine)
XVDLDI